European Patent Specification EP 3 690 054 B1, published December 11, 2024. Title: PHARMACEUTICAL COMPOSITION FOR PREVENTING OR TREATING HEART FAILURE. Applicant: BethphaGen Inc. The sequence listing filed with the application follows.

SEQUENCE LISTING (14 sequences)

SEQ ID NO: 1 - protein, 997 aa, Homo sapiens
MENAHTKTVEEVLGHFGVNESTGLSLEQVKKLKERWGSNELPAEEGKTLLELVIEQFEDLLVRILLLAACISFVLAWFEEGEETITAFVEPFVILLILVANAIVGVWQERNAENAIEALKEYEPEMGKVYRQDRKSVQRIKAKDIVPGDIVEIAVGDKVPADIRLTSIKSTTLRVDQSILTGESVSVIKHTDPVPDPRAVNQDKKNMLFSGTNIAAGKAMGVVVATGVNTEIGKIRDEMVATEQERTPLQQKLDEFGEQLSKVISLICIAVWIINIGHFNDPVHGGSWIRGAIYYFKIAVALAVAAIPEGLPAVITTCLALGTRRMAKKNAIVRSLPSVETLGCTSVICSDKTGTLTTNQMSVCRMFILDRVEGDTCSLNEFTITGSTYAPIGEVHKDDKPVNCHQYDGLVELATICALCNDSALDYNEAKGVYEKVGEATETALTCLVEKMNVFDTELKGLSKIERANACNSVIKQLMKKEFTLEFSRDRKSMSVYCTPNKPSRTSMSKMFVKGAPEGVIDRCTHIRVGSTKVPMTSGVKQKIMSVIREWGSGSDTLRCLALATHDNPLRREEMHLEDSANFIKYETNLTFVGCVGMLDPPRIEVASSVKLCRQAGIRVIMITGDNKGTAVAICRRIGIFGQDEDVTSKAFTGREFDELNPSAQRDACLNARCFARVEPSHKSKIVEFLQSFDEITAMTGDGVNDAPALKKAEIGIAMGSGTAVAKTASEMVLADDNFSTIVAAVEEGRAIYNNMKQFIRYLISSNVGEVVCIFLTAALGFPEALIPVQLLWVNLVTDGLPATALGFNPPDLDIMNKPPRNPKEPLISGWLFFRYLAIGCYVGAATVGAAAWWFIAADGGPRVSFYQLSHFLQCKEDNPDFEGVDCAIFESPYPMTMALSVLVTIEMCNALNSLSENQSLLRMPPWENIWLVGSICLSMSLHFLILYVEPLPLIFQITPLNVTQWLMVLKISLPVILMDETLKFVARNYLEPAILE

SEQ ID NO: 2 - DNA, 2991 bp, Homo sapiens
atggagaacgcgcacaccaagacggtggaggaggtgctgggccacttcggcgtcaacgagagtacggggctgagcctggaacaggtcaagaagcttaaggagagatggggctccaacgagttaccggctgaagaaggaaaaaccttgctggaacttgtgattgagcagtttgaagacttgctagttaggattttattactggcagcatgtatatcttttgttttggcttggtttgaagaaggtgaagaaacaattacagcctttgtagaaccttttgtaattttactcatattagtagccaatgcaattgtgggtgtatggcaggaaagaaatgctgaaaatgccatcgaagcccttaaggaatatgagcctgaaatgggcaaagtgtatcgacaggacagaaagagtgtgcagcggattaaagctaaagacatagttcctggtgatattgtagaaattgctgttggtgacaaagttcctgctgatataaggttaacttccatcaaatctaccacactaagagttgaccagtcaattctcacaggtgaatctgtctctgtcatcaagcacactgatcccgtccctgacccacgagctgtcaaccaagataaaaagaacatgctgttttctggtacaaacattgctgctgggaaagctatgggagtggtggtagcaactggagttaacaccgaaattggcaagatccgggatgaaatggtggcaacagaacaggagagaacaccccttcagcaaaaactagatgaatttggggaacagctttccaaagtcatctcccttatttgcattgcagtctggatcataaatattgggcacttcaatgacccggttcatggagggtcctggatcagaggtgctatttactactttaaaattgcagtggccctggctgtagcagccattcctgaaggtctgcctgcagtcatcaccacctgcctggctcttggaactcgcagaatggcaaagaaaaatgccattgttcgaagcctcccgtctgtggaaacccttggttgtacttctgttatctgctcagacaagactggtacacttacaacaaaccagatgtcagtctgcaggatgttcattctggacagagtggaaggtgatacttgttcccttaatgagtttaccataactggatcaacttatgcacctattggagaagtgcataaagatgataaaccagtgaattgtcaccagtatgatggtctggtagaattagcaacaatttgtgctctttgtaatgactctgctttggattacaatgaggcaaagggtgtgtatgaaaaagttggagaagctacagagactgctctcacttgcctagtagagaagatgaatgtatttgataccgaattgaagggtctttctaaaatagaacgtgcaaatgcctgcaactcagtcattaaacagctgatgaaaaaggaattcactctagagttttcacgtgacagaaagtcaatgtcggtttactgtacaccaaataaaccaagcaggacatcaatgagcaagatgtttgtgaagggtgctcctgaaggtgtcattgacaggtgcacccacattcgagttggaagtactaaggttcctatgacctctggagtcaaacagaagatcatgtctgtcattcgagagtggggtagtggcagcgacacactgcgatgcctggccctggccactcatgacaacccactgagaagagaagaaatgcaccttgaggactctgccaactttattaaatatgagaccaatctgaccttcgttggctgcgtgggcatgctggatcctccgagaatcgaggtggcctcctccgtgaagctgtgccggcaagcaggcatccgggtcatcatgatcactggggacaacaagggcactgctgtggccatctgtcgccgcatcggcatcttcgggcaggatgaggacgtgacgtcaaaagctttcacaggccgggagtttgatgaactcaacccctccgcccagcgagacgcctgcctgaacgcccgctgttttgctcgagttgaaccctcccacaagtctaaaatcgtagaatttcttcagtcttttgatgagattacagctatgactggcgatggcgtgaacgatgctcctgctctgaagaaagccgagattggcattgctatgggctctggcactgcggtggctaaaaccgcctctgagatggtcctggcggatgacaacttctccaccattgtggctgccgttgaggaggggcgggcaatctacaacaacatgaaacagttcatccgctacctcatctcgtccaacgtcggggaagttgtctgtattttcctgacagcagcccttggatttcccgaggctttgattcctgttcagctgctctgggtcaatctggtgacagatggcctgcctgccactgcactggggttcaaccctcctgatctggacatcatgaataaacctccccggaacccaaaggaaccattgatcagcgggtggctctttttccgttacttggctattggctgttacgtcggcgctgctaccgtgggtgctgctgcatggtggttcattgctgctgacggtggtccaagagtgtccttctaccagctgagtcatttcctacagtgtaaagaggacaacccggactttgaaggcgtggattgtgcaatctttgaatccccatacccgatgacaatggcgctctctgttctagtaactatagaaatgtgtaacgccctcaacagcttgtccgaaaaccagtccttgctgaggatgcccccctgggagaacatctggctcgtgggctccatctgcctgtccatgtcactccacttcctgatcctctatgtcgaacccttgccactcatcttccagatcacaccgctgaacgtgacccagtggctgatggtgctgaaaatctccttgcccgtgattctcatggatgagacgctcaagtttgtggcccgcaactacctggaacctgcaatactggag

SEQ ID NO: 3 - protein, 250 aa, Homo sapiens
MRGTPKTHLLAFSLLCLLSKVRTQLCPTPCTCPWPPPRCPLGVPLVLDGCGCCRVCARRLGEPCDQLHVCDASQGLVCQPGAGPGGRGALCLLAEDDSSCEVNGRLYREGETFQPHCSIRCRCEDGGFTCVPLCSEDVRLPSWDCPHPRRVEVLGKCCPEWVCGQGGGLGTQPLPAQGPQFSGLVSSLPPGVPCPEWSTAWGPCSTTCGLGMATRVSNQNRFCRLETQRRLCLSRPCPPSRGRSPQNSAF

SEQ ID NO: 4 - DNA, 750 bp, Homo sapiens
atgagaggcacaccgaagacccacctcctggccttctccctcctctgcctcctctcaaaggtgcgtacccagctgtgcccgacaccatgtacctgcccctggccacctccccgatgcccgctgggagtacccctggtgctggatggctgtggctgctgccgggtatgtgcacggcggctgggggagccctgcgaccaactccacgtctgcgacgccagccagggcctggtctgccagcccggggcaggacccggtggccggggggccctgtgcctcttggcagaggacgacagcagctgtgaggtgaacggccgcctgtatcgggaaggggagaccttccagccccactgcagcatccgctgccgctgcgaggacggcggcttcacctgcgtgccgctgtgcagcgaggatgtgcggctgcccagctgggactgcccccaccccaggagggtcgaggtcctgggcaagtgctgccctgagtgggtgtgcggccaaggagggggactggggacccagccccttccagcccaaggaccccagttttctggccttgtctcttccctgccccctggtgtcccctgcccagaatggagcacggcctggggaccctgctcgaccacctgtgggctgggcatggccacccgggtgtccaaccagaaccgcttctgccgactggagacccagcgccgcctgtgcctgtccaggccctgcccaccctccaggggtcgcagtccacaaaacagtgccttc

SEQ ID NO: 5 - protein, 22 aa, Artificial Sequence
  self-cleavage sequence derived from porcine teschovirus-1
GSGATNFSLLKQAGDVEENPGP

SEQ ID NO: 6 - DNA, 66 bp, Artificial Sequence
  self-cleavage sequence derived from porcine teschovirus-1
ggaagcggagctactaacttcagcctgctgaagcaggctggagacgtggaggagaaccctggacct

SEQ ID NO: 7 - protein, 21 aa, Artificial Sequence
  self-cleavage sequence derived from Thoseaasigna virus
GSGEGRGSLLTCGDVEENPGP

SEQ ID NO: 8 - DNA, 63 bp, Artificial Sequence
  self-cleavage sequence derived from Thoseaasigna virus
ggaagcggagagggcagaggaagtctgctaacatgcggtgacgtcgaggagaatcctggacct

SEQ ID NO: 9 - protein, 23 aa, Artificial Sequence
  self-cleavage sequence derived from equine rhinitis A virus (ERAV)
GSGQCTNYALLKLAGDVESNPGP

SEQ ID NO: 10 - DNA, 69 bp, Artificial Sequence
  self-cleavage sequence derived from equine rhinitis A virus (ERAV)
ggaagcggacagtgtactaattatgctctcttgaaattggctggagatgttgagagcaaccctggacct

SEQ ID NO: 11 - protein, 25 aa, Artificial Sequence
  self-cleavage sequence derived from FMDV 2A
GSGVKQTLNFDLLKLAGDVESNPGP

SEQ ID NO: 12 - DNA, 75 bp, Artificial Sequence
  self-cleavage sequence derived from FMDV 2A
ggaagcggagtgaaacagactttgaattttgaccttctcaagttggcgggagacgtggagtccaaccctggacct

SEQ ID NO: 13 - DNA, 2994 bp, Homo sapiens
atggagaacgcgcacaccaagacggtggaggaggtgctgggccacttcggcgtcaacgagagtacggggctgagcctggaacaggtcaagaagcttaaggagagatggggctccaacgagttaccggctgaagaaggaaaaaccttgctggaacttgtgattgagcagtttgaagacttgctagttaggattttattactggcagcatgtatatcttttgttttggcttggtttgaagaaggtgaagaaacaattacagcctttgtagaaccttttgtaattttactcatattagtagccaatgcaattgtgggtgtatggcaggaaagaaatgctgaaaatgccatcgaagcccttaaggaatatgagcctgaaatgggcaaagtgtatcgacaggacagaaagagtgtgcagcggattaaagctaaagacatagttcctggtgatattgtagaaattgctgttggtgacaaagttcctgctgatataaggttaacttccatcaaatctaccacactaagagttgaccagtcaattctcacaggtgaatctgtctctgtcatcaagcacactgatcccgtccctgacccacgagctgtcaaccaagataaaaagaacatgctgttttctggtacaaacattgctgctgggaaagctatgggagtggtggtagcaactggagttaacaccgaaattggcaagatccgggatgaaatggtggcaacagaacaggagagaacaccccttcagcaaaaactagatgaatttggggaacagctttccaaagtcatctcccttatttgcattgcagtctggatcataaatattgggcacttcaatgacccggttcatggagggtcctggatcagaggtgctatttactactttaaaattgcagtggccctggctgtagcagccattcctgaaggtctgcctgcagtcatcaccacctgcctggctcttggaactcgcagaatggcaaagaaaaatgccattgttcgaagcctcccgtctgtggaaacccttggttgtacttctgttatctgctcagacaagactggtacacttacaacaaaccagatgtcagtctgcaggatgttcattctggacagagtggaaggtgatacttgttcccttaatgagtttaccataactggatcaacttatgcacctattggagaagtgcataaagatgataaaccagtgaattgtcaccagtatgatggtctggtagaattagcaacaatttgtgctctttgtaatgactctgctttggattacaatgaggcaaagggtgtgtatgaaaaagttggagaagctacagagactgctctcacttgcctagtagagaagatgaatgtatttgataccgaattgaagggtctttctaaaatagaacgtgcaaatgcctgcaactcagtcattaaacagctgatgaaaaaggaattcactctagagttttcacgtgacagaaagtcaatgtcggtttactgtacaccaaataaaccaagcaggacatcaatgagcaagatgtttgtgaagggtgctcctgaaggtgtcattgacaggtgcacccacattcgagttggaagtactaaggttcctatgacctctggagtcaaacagaagatcatgtctgtcattcgagagtggggtagtggcagcgacacactgcgatgcctggccctggccactcatgacaacccactgagaagagaagaaatgcaccttgaggactctgccaactttattaaatatgagaccaatctgaccttcgttggctgcgtgggcatgctggatcctccgagaatcgaggtggcctcctccgtgaagctgtgccggcaagcaggcatccgggtcatcatgatcactggggacaacaagggcactgctgtggccatctgtcgccgcatcggcatcttcgggcaggatgaggacgtgacgtcaaaagctttcacaggccgggagtttgatgaactcaacccctccgcccagcgagacgcctgcctgaacgcccgctgttttgctcgagttgaaccctcccacaagtctaaaatcgtagaatttcttcagtcttttgatgagattacagctatgactggcgatggcgtgaacgatgctcctgctctgaagaaagccgagattggcattgctatgggctctggcactgcggtggctaaaaccgcctctgagatggtcctggcggatgacaacttctccaccattgtggctgccgttgaggaggggcgggcaatctacaacaacatgaaacagttcatccgctacctcatctcgtccaacgtcggggaagttgtctgtattttcctgacagcagcccttggatttcccgaggctttgattcctgttcagctgctctgggtcaatctggtgacagatggcctgcctgccactgcactggggttcaaccctcctgatctggacatcatgaataaacctccccggaacccaaaggaaccattgatcagcgggtggctctttttccgttacttggctattggctgttacgtcggcgctgctaccgtgggtgctgctgcatggtggttcattgctgctgacggtggtccaagagtgtccttctaccagctgagtcatttcctacagtgtaaagaggacaacccggactttgaaggcgtggattgtgcaatctttgaatccccatacccgatgacaatggcgctctctgttctagtaactatagaaatgtgtaacgccctcaacagcttgtccgaaaaccagtccttgctgaggatgcccccctgggagaacatctggctcgtgggctccatctgcctgtccatgtcactccacttcctgatcctctatgtcgaacccttgccactcatcttccagatcacaccgctgaacgtgacccagtggctgatggtgctgaaaatctccttgcccgtgattctcatggatgagacgctcaagtttgtggcccgcaactacctggaacctgcaatactggagtag

SEQ ID NO: 14 - DNA, 753 bp, Homo sapiens
atgagaggcacaccgaagacccacctcctggccttctccctcctctgcctcctctcaaaggtgcgtacccagctgtgcccgacaccatgtacctgcccctggccacctccccgatgcccgctgggagtacccctggtgctggatggctgtggctgctgccgggtatgtgcacggcggctgggggagccctgcgaccaactccacgtctgcgacgccagccagggcctggtctgccagcccggggcaggacccggtggccggggggccctgtgcctcttggcagaggacgacagcagctgtgaggtgaacggccgcctgtatcgggaaggggagaccttccagccccactgcagcatccgctgccgctgcgaggacggcggcttcacctgcgtgccgctgtgcagcgaggatgtgcggctgcccagctgggactgcccccaccccaggagggtcgaggtcctgggcaagtgctgccctgagtgggtgtgcggccaaggagggggactggggacccagccccttccagcccaaggaccccagttttctggccttgtctcttccctgccccctggtgtcccctgcccagaatggagcacggcctggggaccctgctcgaccacctgtgggctgggcatggccacccgggtgtccaaccagaaccgcttctgccgactggagacccagcgccgcctgtgcctgtccaggccctgcccaccctccaggggtcgcagtccacaaaacagtgccttctag